European Patent Application EP 4 685 234 A2, published January 28, 2026. Title: PROTEASES FOR BEER HAZE REDUCTION. Applicant: International N&H Denmark ApS. Application EP 25222183.3, filed June 17, 2022. The sequence listing filed with the application follows.

SEQUENCE LISTING (16 sequences)

SEQ ID NO: 1 - protein, 527 aa, Aspergillus bertholletius
MHFLAPLSVVTLLASWPLLGYAIHPPKPVPPPVSRPVSTRSSAVVGEATFDQLLDHHDSSKGTFSQRYWWSTEYWGGPGSPVVLFTPGEASADGYQGYLTNTTLTGRYAQEIQGAVILIEHRYWGGSSPYKELTAETLQYLTLEQSILDLTYFAETVSLEFDPSNRSNAPKAPWVLVGGSYSGALAAWTAAVAPETFWAYHATSAPVEAINDFWQYFDPIRQGMAPNCSRDVSLVATHIDRVGKHGSAAEQLALKELFGLGAVEHYDDFAAALPIGPYKWQSNTFVTGYSGFFAFCDAVENVKAGATVVPGPEGVGLQKALRGYAKWFKSTILPGYCANYGYWTDNQTVACFDTYNPSSAIFTDTSVDNAVDRQWQWFLCNEPFFWWQDGAPEGIPTIIPRTVNAAYWQRQCSLYFPEVNGYTYGSAKGKTAATVNQWTGGWSATRNTSHLLWVNGQYDPWRDSGVSSIYRPGGPLKSTADEPVQVIPGGFHCSDLYLKDYYANDGVKQVIDNAVAQIKSWVAEYYN

SEQ ID NO: 2 - protein, 524 aa, Aspergillus niger
MQTFGAFLVSFLAASGLAAAARPRLVPKPISRPASSKSAATTGEAYFEQLLDHHNPEKGTFSQRYWWSTEYWGGPGSPVVLFNPGEVSADGYEGYLTNDTLTGVYAQEIQGAVILIEHRYWGDSSPYEVLNAETLQYLTLDQSILDMTYFAETVKLQFDNSSRSNAQNAPWVMVGGSYSGALTAWTESIAPGTFWAYHATSAPVEAIYDFWQYFYPIQQGMAQNCSKDVSLVAEYVDKIGKNGTAKEQQELKELFGLGAVEHYDDFAAVLPNGPYLWQDNDFVTGYSSFFQFCDAVEGVEAGAAVTPGPEGVGLEKALANYANWFNSTILPNYCASYGYWTDEWSVACFDSYNASSPIFTDTSVGNPVDRQWEWFLCNEPFFWWQDGAPEGTSTIVPRLVSASYWQRQCPLYFPEVNGYTYGSAKGKNSATVNSWTGGWDMTRNTTRLIWTNGQYDPWRDSGVSSTFRPGGPLVSTANEPVQIIPGGFHCSDLYMEDYYANEGVRKVVDNEVKQIKEWVEEYYA

SEQ ID NO: 3 - protein, 527 aa, Aspergillus transmontanensis
MQFLPPLSIVTLLASWPSLSRAIHPPRPVPPPVSRPVSTQSLAVEGNATFEQLLDHHDSSKGTFSQRYWWSTEYWGGPGSPVVLFTPGEASADGYEGYLTNNTLTGLYAQEIQGAVILIEHRYWGDSSPYEELTAETLQYLTLEQSILDLTHFAETVQLEFDTSNSSNAPKAPWVLVGGSYSGALAAWTAAVAPETFWAYHATSAPVQAIDDFWQYFDPIRHGMAPNCSRDVSLVANHIDTVGKNGSAADQFALKELFGLEALEHYDDFAAALPTGPYLWQSNTFVTGYSDFFAFCDAVENVEAGAAVVPGPEGVGLQKALTGYANWFNSTILPGYCASYGYWTDNRTVACFDTHNPSSAIFIDTSVDNAVDRQWQWFLCNEPFFWWQDGAPEGVPTIVPRTINAEYWQRQCSLYFPEVNGYTYGSAKGKTAASVNSWTGGWSDSKNTSRLLWVNGQYDPWRDSGVSSTHRPGGPLASTADEPVQIIPGGFHCSDLYIKDYYANAGVKQVVDNAVAQIKSWVAEYYK

SEQ ID NO: 4 - protein, 525 aa, Aspergillus homomorphus
MRFCSPVSVVAVTALWASLTAALRPPRLAPRPVTATTQSAVVESTFEQLIDHNDPSKGTFSQRYWYSTQYWGGPGSPVVLFTPGEAAADGYGGYLTNRTLTGVYAQQLQGAVVLIEHRYWGGSSPYANLTAETLQYLTLEQSVLDLTYFAENVQLGFAKNSTSSNAPHVPWVLVGGSYSGALTAWTEHLAPGTFWAYHATSAPMESIYDFWTYFRPIQEGMAKNCSKDVSLVAEHVDKVGKLGTKAQQKALKKLFGLEALEHFDDFAAVLPIGPYLWQDNSFATGYSGFFAFCDAVENVEAGAAVTPGAEGVGLEKALKGYANWFKNKILPDYCASTYGYWSDKYTVACFDTYNATSPLFRDTSVRNAVDRQWTWFLCNEPFFWWQDGAPESETSLIPRLVSADYWQRQCSLYFPEVNGYTYGSAKGKTASTFNAWTDGWFLTGNSTRLIWTNGQYDPWRDAGVSSIFRPGGPLVSTPNEPVQIIPGGFHCSDLYISDAEVNAGVKKVVINEVAQIKAWVAEFYA

SEQ ID NO: 5 - protein, 524 aa, Aspergillus pseudocaelatus
MHFLSRISVVTLLASWPSLSRAIHPPRPVPPPVTRPASTLSSAVEGEATFEQLVDHHDSSKGTFSQRYWWSTEYWGGPGSPVVLFTPGEASADGYEGYLTNNTLTGLYAQEIQGAVILIEHRYWGGSSPFEELTAETLQYLTLEQSIQDLTYFAETVQLEFDTSNSSNAPKAPWVLVGGSYSGALAAWTAAVAPETFWAYHATSAPVQAINDFWQYFDPIRHGMAPNCSRDVSLVANHIDSVGKNGSIAEQSALKELFGLGALEHYDDFAAALPIGPYLWQDNTFVTGYSGFFAFCDAVENVEAGAAVVPGPEGVGLQKALTGYANWFNSTILPGYCANYGYWTDNRTVACFDTHNSSSAIFTDTSLNNAVDRQWQWFLCNEPFFWWQDGAPEGVPSIVPRTVNAAYWQRQCSLYFPEVNGYTYGSAKGKTAATVNTWTGGWSETKNTSHLLWVNGQYDPWRDSGVSSTHRPGGPLASTADEPVQVIPGGFHCSDLYLKDYHANAGVKQVVDNAVAQIKSWVAE

SEQ ID NO: 6 - protein, 526 aa, Aspergillus neoauricomus
MRFLSVVRLAALVTSWASIAQAIRPPIPVPEPVPRPVSLQSTSTQGQATFQQLLDHHDPSKGTFSQRYWWSTEFWGGPGSPVILFTPGEVAADGYQGYLTNKTLTGHYAQEVQAAVVLVEHRYWGGSSPYKNLTAETLQYLTLEQSILDFTHFAKTVQLQFDNSTRSNAQRAPWVFVGGSYSGALAAWTEATAPGTFWAYHATSAPVEAIYDFWQYFEPVREGMPQNCSKDVSLVANYIDGLGKNGTTREKQAVKELFGLGDLEYYDDFAAIFPIGPWSWQSNSFITGYSDFYQFCDSVENVKAGAPVVPGPEGVGLLKALAGYAKWFNSTALPGYCASYGYWTDERSISCFDTHNASSPLFTDTSVANGMDRQWQWFLCNEPFFYWQDGAPEGKTTIVPRTVSAEYWQRQCPLFFPTVNGHTYGSAKGKNAATVNAYTGGWSRTNTSRLIWTNGQYDPWLDSGVSSRFRPGGPLESTAAAPVQVIPGGFHCSDLYMTSYAVNDGVKKVVDNEVAQIKAWIGEYYK

SEQ ID NO: 7 - protein, 524 aa, Aspergillus albertensis
MHFASSARAVALLASLTHAIRPPRPVPPPVSGPVSAQLSAVGGQATFEQLLDHHDASKGVFSQRYWWSTEYWGGPGSPVVLFTPGESAADGYEGYLTNNTLTGLYAQEIQGAVVLIEHRYWGESSPYDQLTAETLQHLTLEQSILDLTYFAENVNLEFDTTNSSNAQDAPWVLVGGSYSGALAAWTEAVAPGTFWAYHATSAPVQAIYDFWQYFDPIRHGMAPNCSRDVSLVANHVDNVGKNGSATQQQALKELFGLGALEHYDDFAAVLPLGPWEWQSNTFVTGYSRFFAFCDAVENVEAGAAAVPGPEGVGLQKALTGYAKWFKSTILPGYCANYGYWTDKMSVACFDTHDKSSPLFTDTSVKNAMDRQWQWFLCNEPFFWWQDGAPEGVPTIVPRTVDAAYWQRQCSLFFPEVNGFTYGSAKGKTADTVNDWTGGWSDTNNSTHLLWVNGQYDPWLDSGVSSTYRPGGPLKSTAEAPVLVIPGSFHCSDLNLKNYYANSGVKQVVDSAVAQIKSWVDEYYK

SEQ ID NO: 8 - protein, 527 aa, Aspergillus coremiiformis
MHFASPLRVVAFLASWPLLTHAFRPPRPVPLPVSRPDSTQLLTAGGQATFEQLLDHHDPSKGTFAQRYWWSTEHWGGPGSPVILFTPGESAADGYGGYLTNNTLTGLYAQEIQGAVILIEHRYWGDSSPYKELTAETLQYLTLEQSILDLTHFAQTVNLEFDPSNRSTASKAPWVLVGGSYSGALTAWTEAIAPGTFWAYHATSAPVEAVYDFWQYFDPIRHGMAPNCSRDVSLVANYVDGVGRNGSATEKQALKELFGLGALEHYDDFAAVLPAGPYLWQSNTFTTGYSDFFAFCDAVENVEAGAAIVPGPEGVGLQKALMGYANWFNSTILPGHCADYGYWTDTWSVACYDTYDPHGALFADTSVRNAADRQWQWFLCNEPFFWWQDGAPEGVPTIVPRTVDAAYWQRQCSLFFPEVNGYTYGSAKGKTAATVNDWTGGWFETKNTTRLLWVNGQYDPWRSSGVSSINRPGGPLQSTPNEPVQVIPGGFHCSDLYMNDYHANPGLKTVVDNAVTQIRSWVAEYYK

SEQ ID NO: 9 - protein, 525 aa, Aspergillus wentii
MRFSAVALLASCTWASLATAIRPPKPVPRPVSRPVSRQSSTFEGQATFDQLLDHHHPEKGTFSQRYWWSTEFWGGPGSPVVLFTPGEESADGYEGYLTNNTLTGVYAQEIQGAVILIEHRYWGGSSPYENLTAETLQYLTLEQSILDLTYFAKTVKLEFDFNGSSNAQKAPWVLVGGSYSGALTAWTEAISPGTFWAYHATSAPVEAIYDFWQYFYPIQQGMAQNCSKDVSLVAEYIDHVGKTGSAKEQQDIKELFGLGALEHYNDFAAVLPIGPYLWQENTFSSGYSDFFQFCDSVENVEAGAAVVPGPEGVGLEKALKGYAKWFNTTMLPGYCADYGYWKDEWSVACFDTHNASSPLFTDTSVENQMDRQWQWFLCNEPFFWWQDGAPENVSTIVPRTVDAAYWQRQCSLFFPETNGYKYGSAKNKTASTVNDWTDGWFLTKNTTRLIWTNGQYDPWRDSGVSSAFRPGGPLVSTPNEPVQIIPGGFHCSDLYIKDATANAGVKKVVDTEVAQIKAWVDEYYK

SEQ ID NO: 10 - protein, 526 aa, Aspergillus brasiliensis
MRSFSAVAAAALALSWASLAQAARPRLAPKPISRPASSKSAATTGKAYFEQLLDHHNPEKGTFSQRYWWSTEYWGGPGSPVVLFTPGEVSADGYEGYLTNETLTGVYAQEIQGAVILIEHRYWGDSSPYDVLNAETLQYLTLDQSILDMTYFAETVKLQFDNSSRSNAQNAPWVMVGGSYSGALTAWTESIAPGTFWAYHATSAPVEAIYDFWQYFYPIQQGMAQNCSKDVSLVAEYVDKVGKNGTAKEQQALKEKFGLGALEHYDDFAAVLPNGPYLWQDNDFATGYSSFFEFCDAIEGVEAGAAVTPGPEGVGLEKALANYANWFNSTILPDYCASYGYWTDEWSVACFDSYNASSPLFTDTSVDNAVDRQWEWFLCNEPFFWWQDGAPEGTSTIVPRLVSASYWQRQCPLYFPEVNGYTYGSAKGKNSATVNSWTGGWDMTRNTTRLIWTNGQYDPWRDSGVSSTFRPGGPLVSTANEPVQVIPGGFHCSDLYMQDYYVNEGVRKVVNNEVKQIKEWVEEYYA

SEQ ID NO: 11 - protein, 526 aa, Aspergillus sclerotioniger
MRSFSAVAAAALAVSWASLAQAARPRLAPKPVSRPASSTSAATTGEAYFEQLVDHHNPEKGTFSQRYWWSTEYWGGPGSPVVLFTPGEVSADGYEGYLTNETLTGVYAQEIQGAVILIEHRYWGDSSPYEVLNAETLQYLTLDQAVLDMTYFAETVKFQFDNSTRSNAQNAPWVMVGGSYSGALTAWVESVAPGTFWAYHATSAPVEAIYDFWQYFYPISQGMAQNCSKDVSLVAEHVDKVGKTGTAEEQQKLKELFGLGALEHYDDFAAVLPNGPYLWQDNDFVTGYSEFFQFCDAVEGVEAGAAVTPGPEGVGLEKALANYANWFNSTMLPNYCASYGYWSDEWSVACFDSYNASSPLFTDTSVGNAVDRQWEWFLCNEPFFWWQDGAPENVTTIVPRLVSAEYWQRQCSLYFPETNGYTFGSAQNKTAATVNDWTGGWFETRNTTRLIWTNGQYDPWRDSGVSSTFRPGGQLVSTANEPVQIIPGGFHCSDLYMEDYYANAGVRKVVDNEVAQIKKWVAEYYA

SEQ ID NO: 12 - DNA, 1790 bp, Magnaporthe oryzae
  source 1..1790: mol_type = genomic DNA
atgctgttcctttcttctctccttctcctggccctgtccggggctccggcctacgcagtccgcgtcggcaaccttttggagccgcctatgcccccgccctttgccatcgaggatatcgaggatatagaccccaagcaacttaccaagcgtaagatcagcagcgggttctttgatcaatacatcgaccacagcaatccttcattgggcacgtttcggcagaagttttggtggagtgatgagttctacaagggtccaggctctcctgtgattctgttcaacccaggagaatcaagggccgatatctacaccggctacctgacgaaccttaccgttcccggcatgtatgcgcaggctgttggtgccgccgtcgtcatgctcgagcaccgctactggggagagtcgtcacctttcgcaaacctcagcaccaagaacatgcagtatctgaccctcaacaactccatctccgatacaactcgctttgcccgccaggtgaagctgccttttgacaccagcggggcgaccaatgcccccaatgctccgtgggtctttgttggtggttcataccctggtgcccttgccggatgggtagagagcgtcgcccctggaactttctgggcctaccatgcgtcaagcgccgtggtccaggatatcggtgattactggcgctactttagcccaattaatgaaggcatgcccaagaactgcagcgccgacatcggccgggtcgtcgagcacattgacaaagtattgggcactggatcagacagcgacaagtctgccctgcagacagcttttggccttggatccctcgagcatgatgactttgtcgagactctggcgaacggcccatacctgtggcagggcattgatttcagcactggctactcggactttttcaagttctgtgactatgttgaggtatgctcgctatcgcctatcctctttgttaaaattggcaggaaactgtggcgcagtaatttgctgacttcatcctctagaacgtacccccgaaagcagcgacaagagtgcccccaggagttgatggtgttggtcttgagaaggcattgacgggctaccaggattggatcaagaaggaatacctcccaaccgcctgcgacagcttgggataccccaagggtgacctgggctgcctgagcagccacaacttctcagcccccttctaccgtgaccagacagtattaaacccggggaaccggcagtggttttggtttctttgcaatgaaccgtgagtggcgacggcagtgggctttgatttaaacttactactgtcttcttttgtactgacacgagtttgcccatccttcagcttcaagttttggcaaaacggcgcccccaagggcgagccgtcgattgtttcgcgtatcataggcagcaaatactttgagagccagtgtgcgttgtggttccccgacgagccgcgtgaaggcggtggcgtttacacgtacggcatcgccgagggcaaggatgtcgccagtgtcaacaaattcaccggtgggtgggaccacaccgacacgaaacgacttctttgggtcaacggccagtttgacccatggctgcacgctacagtgtcgtcgccctcccgccccggaggtccccttcaatcgacagacaaggcacctgttctggttatcccgggtggagtacactgcaccgacttgattatacgcaacggagacgccaacgagggcgcgcgcaaggtccagagtcaggcacgcgaaatcatcaagaaatgggtgtccgagtttcccaagagcggaaagagcccttga

SEQ ID NO: 13 - protein, 542 aa, Magnaporthe oryzae
MLFLSSLLLLALSGAPAYAVRVGNLLEPPMPPPFAIEDIEDIDPKQLTKRKISSGFFDQYIDHSNPSLGTFRQKFWWSDEFYKGPGSPVILFNPGESRADIYTGYLTNLTVPGMYAQAVGAAVVMLEHRYWGESSPFANLSTKNMQYLTLNNSISDTTRFARQVKLPFDTSGATNAPNAPWVFVGGSYPGALAGWVESVAPGTFWAYHASSAVVQDIGDYWRYFSPINEGMPKNCSADIGRVVEHIDKVLGTGSDSDKSALQTAFGLGSLEHDDFVETLANGPYLWQGIDFSTGYSDFFKFCDYVENVPPKAATRVPPGVDGVGLEKALTGYQDWIKKEYLPTACDSLGYPKGDLGCLSSHNFSAPFYRDQTVLNPGNRQWFWFLCNEPFKFWQNGAPKGEPSIVSRIIGSKYFESQCALWFPDEPREGGGVYTYGIAEGKDVASVNKFTGGWDHTDTKRLLWVNGQFDPWLHATVSSPSRPGGPLQSTDKAPVLVIPGGVHCTDLIIRNGDANEGARKVQSQAREIIKKWVSEFPKSGKSP

SEQ ID NO: 14 - protein, 523 aa, Magnaporthe oryzae
VRVGNLLEPPMPPPFAIEDIEDIDPKQLTKRKISSGFFDQYIDHSNPSLGTFRQKFWWSDEFYKGPGSPVILFNPGESRADIYTGYLTNLTVPGMYAQAVGAAVVMLEHRYWGESSPFANLSTKNMQYLTLNNSISDTTRFARQVKLPFDTSGATNAPNAPWVFVGGSYPGALAGWVESVAPGTFWAYHASSAVVQDIGDYWRYFSPINEGMPKNCSADIGRVVEHIDKVLGTGSDSDKSALQTAFGLGSLEHDDFVETLANGPYLWQGIDFSTGYSDFFKFCDYVENVPPKAATRVPPGVDGVGLEKALTGYQDWIKKEYLPTACDSLGYPKGDLGCLSSHNFSAPFYRDQTVLNPGNRQWFWFLCNEPFKFWQNGAPKGEPSIVSRIIGSKYFESQCALWFPDEPREGGGVYTYGIAEGKDVASVNKFTGGWDHTDTKRLLWVNGQFDPWLHATVSSPSRPGGPLQSTDKAPVLVIPGGVHCTDLIIRNGDANEGARKVQSQAREIIKKWVSEFPKSGKSP

SEQ ID NO: 15 - DNA, 1629 bp, synthetic construct
  misc_feature 1..1629: note = Synthesized
  source 1..1629: mol_type = other DNA
atgctctttctgagctccctcctgctgctcgctctcagcggcgctcccgcctacgccgttcgagttggcaacctcctggagcctcccatgcctcctccctttgctattgaggacatcgaagacattgaccctaagcagctcaccaagcgaaaaatcagcagcggtttcttcgaccagtacatcgaccactccaaccccagcctcggtactttccgccaaaagttttggtggtccgacgagttctacaagggccccggttcccccgtcatcctgttcaaccctggcgaaagccgcgctgatatctacaccggctatctgactaacctcaccgtccccggcatgtacgctcaagccgtcggtgctgccgttgtcatgctggagcaccgctattggggcgagtccagccccttcgccaatctctccaccaagaacatgcagtacctgaccctcaacaacagcattagcgacaccacccgctttgcccgccaggtcaagctgccctttgacacctccggcgccaccaatgctcctaatgccccctgggtctttgtcggtggtagctatcctggtgccctggccggttgggtcgagagcgttgctcctggcaccttctgggcctatcatgccagctccgccgtcgttcaagatatcggcgactattggcgctactttagccccatcaacgagggcatgcctaaaaactgcagcgccgacatcggtcgcgtcgtcgaacacatcgataaggtcctgggtaccggctccgacagcgataagagcgccctgcagaccgctttcggcctcggcagcctggaacacgacgacttcgtcgagaccctcgccaacggcccctacctctggcagggcatcgacttcagcactggctacagcgacttcttcaagttctgcgactacgtcgagaatgtccctcccaaggccgccactcgcgttcctcccggcgtcgacggcgtcggcctggagaaggccctgaccggttaccaggactggatcaagaaggagtacctccccaccgcctgcgattccctcggctaccccaaaggcgatctcggttgcctcagctcccacaacttctccgcccctttctaccgcgatcagaccgtcctcaaccccggtaatcgccagtggttctggttcctctgcaacgagcccttcaagttctggcaaaacggcgcccccaagggcgagcccagcatcgtcagccgcattattggcagcaagtacttcgagtcccagtgcgccctctggtttcccgatgagccccgcgagggcggcggtgtttatacttacggcatcgccgaaggtaaggatgtcgccagcgtcaataagtttactggcggctgggaccatactgacaccaaacgcctcctgtgggttaacggccagttcgacccctggctccacgccactgtcagcagccctagccgacccggtggccccctccagagcactgacaaggcccctgtcctcgttattcccggcggcgtccactgcaccgatctcatcatccgcaacggcgacgctaacgaaggcgctcgcaaggttcaaagccaggcccgcgagatcattaagaagtgggtcagcgagtttcctaaaagcggcaagtccccctaa

SEQ ID NO: 16 - protein, 488 aa, Aspergillus niger
KSAATTGEAYFEQLLDHHNPEKGTFSQRYWWSTEYWGGPGSPVVLFNPGEVSADGYEGYLTNDTLTGVYAQEIQGAVILIEHRYWGDSSPYEVLNAETLQYLTLDQSILDMTYFAETVKLQFDNSSRSNAQNAPWVMVGGSYSGALTAWTESIAPGTFWAYHATSAPVEAIYDFWQYFYPIQQGMAQNCSKDVSLVAEYVDKIGKNGTAKEQQELKELFGLGAVEHYDDFAAVLPNGPYLWQDNDFVTGYSSFFQFCDAVEGVEAGAAVTPGPEGVGLEKALANYANWFNSTILPNYCASYGYWTDEWSVACFDSYNASSPIFTDTSVGNPVDRQWEWFLCNEPFFWWQDGAPEGTSTIVPRLVSASYWQRQCPLYFPEVNGYTYGSAKGKNSATVNSWTGGWDMTRNTTRLIWTNGQYDPWRDSGVSSTFRPGGPLVSTANEPVQIIPGGFHCSDLYMEDYYANEGVRKVVDNEVKQIKEWVEEYYA